European Patent Application EP 4 538 283 A1, published April 16, 2025. Title: L-Histidine Export Protein and Method of Producing L-Histidine Using the Same. Applicant: CJ CheilJedang Corporation. The sequence listing filed with the application follows.

SEQUENCE LISTING (56 sequences)

SEQ ID NO: 1 - protein, 314 aa, synthetic construct
  REGION 1..314: note = synthetic_Haq protein
MKSKNATLVGLSAVVLWSAIVGLIRGVSEHLGATGGAAAIYTVASLILLVSVGFPRLASFPRRYLLWGSVLFVAYELCLSLSIGYAHTGRQAIEVGMVNYLWPTFTLVAAILFGGQRATLLVVPGFILSMLGICWVLGGDQGLDPSGMLANIRDNPLSYGLAFIGALIWAAYCTVTTRIAQGQNGVTPFFMLVALALWVKVLLGGHVAELSFSVPALVYLVLAAAAMGLGYAAWNVGILHGNVTVLAGASYFIPVFSSALSALLLRAPLPTSFWVGAALVCAGSILCWRATRSLDLSKEPAARAARPEGPPQNQ

SEQ ID NO: 2 - DNA, 945 bp, synthetic construct
  misc_feature 1..945: note = synthetic_Haq gene encoding Haq protein
  source 1..945: mol_type = other DNA
atgaagagcaagaacgcaaccctggtcggattgagcgcggtggtactgtggagtgccatcgtgggcctgatccgtggcgtgagcgagcatctcggagccaccggcggggcggcggccatttacacggtggcttcgctgatcctgctggtgtcggtgggattcccgcgcctggcgagtttcccgcgcaggtatctgctatggggcagcgtgctgttcgtggcttatgaattgtgcctgtcgctctcgatcggttatgcccataccggccgccaggccatcgaagtcggcatggtcaattacctctggccgaccttcaccctggtggcggccatcctcttcggaggccagcgcgccacgctgctggtggtgccaggcttcatcctttccatgctgggcatctgctgggtgctcgggggcgaccaggggctggatccttccggcatgctggccaatatccgtgacaatccgctgagctacggcctggccttcatcggggccttgatctgggcggcctactgcaccgtgactacccgcatcgcccaaggccagaacggggtgacgcctttcttcatgctggtggcattggcattgtgggtgaaggtgctgctgggcgggcatgtggctgaactatccttcagtgtgcccgcactggtctacctggtgctggctgcggcggcgatggggctgggctatgcggcctggaacgtgggcatcctgcatggcaatgtgacagtgctggccggtgcctcgtatttcatcccggtcttttcttcggccttgtcggccttgctgctacgtgcgccgctgcccacctcgttctgggtgggcgctgcgctggtgtgcgccgggtcgatcctgtgctggcgggctacccgcagcctggatttgtcaaaagaacctgcagcgcgggcggcacgtcccgaaggcccacctcagaaccaatag

SEQ ID NO: 3 - protein, 312 aa, synthetic construct
  REGION 1..312: note = synthetic_Cpi protein
MQSTRKATLIGLIAILLWSSIVGLIRGVSESLGATGGAAMMYSVASVLLMLTVGFVRLREFPRRYLVWGSILFVSYELCLSLSIGYSHSGRQAIEVGMVNYLWPSFTMLCAIAFNKQKANVLIVPGFLIAILGICLVLGGEQGLDVAGMVANVRDNPLSYGLALAGALIWAAYCTVTNRIAGGNNGVTLFFMLTAMALWIKYFTGDHAPMAFTYHAVIYLALAASAMGFGYPAWNVGILHGNVTVLAGASYFIPVISAALAGLLLHIPLSLAFWKGASLVCAGSVLCWLATRARKVAATPDRAPVRDRVWKQ

SEQ ID NO: 4 - DNA, 939 bp, synthetic construct
  misc_feature 1..939: note = synthetic_Cpi gene encoding Cpi protein
  source 1..939: mol_type = other DNA
atgcaaagcacgcgtaaggccacgttgatcgggctcattgcgatcctgttgtggagttccatcgtcggcctgatccgcggcgtcagtgaaagcctcggcgcgaccggtggcgccgccatgatgtactcggttgcctccgtcctgcttatgctgacggttggcttcgtgcgtctgcgcgaatttccgcggcgctatctggtctggggcagcatcctgttcgtctcctacgaactgtgcctgtcgctgtccatcggctattcgcacagcggcaggcaggcgatcgaggtggggatggtcaattacctctggccgtctttcaccatgttgtgcgccatcgccttcaacaagcagaaggcgaacgttctgatcgtgccgggcttcctgattgcgatcctgggtatctgcctggtgctgggcggcgagcagggtctggatgttgcaggcatggtggccaatgtcagggacaatccgctcagctacggcctcgctttagcgggcgcgctgatctgggcggcctattgcaccgtgaccaacaggattgccggcggcaacaacggcgtcacgctgtttttcatgctcaccgcaatggcgctgtggatcaagtacttcaccggcgaccatgcgccgatggctttcacataccacgccgtcatctacctggcactggcagcgtcggcgatgggcttcggctacccggcgtggaacgtgggcatcctgcacggcaacgtaacggtgcttgccggcgcgtcgtatttcatccctgtgatttcagccgcactggctggcttgctcttgcatataccgctttcgctggcgttctggaaaggcgcgtcgctggtatgcgcggggtccgtgctgtgctggttggcgacgcgcgcgcgcaaggtggctgcaacgcccgaccgtgctccggtccgcgaccgtgtctggaagcaatga

SEQ ID NO: 5 - protein, 293 aa, synthetic construct
  REGION 1..293: note = synthetic_Kcr protein
MDKKRATLIGFSAIILWSTMVGLIRGVSEGLGPVGGAAMIYSLSGLLLIFTVGFPQLRQIPPRYLLVGSLFFVSYEMCLALSLGYAGTRQQAIEVGMVNYLWPSLTILFAIIFNGQKTTWLVIPGLLLSIVGVTWVLGGEHGLDLAEIRSNVISSPLSYILAFVGAFIWAAYCTVTAKYAKGKNGITLFVLFTALALWVKFLMSEQPPMIFSWPVVIKLVTCALALGFAYAAWNVGILHGNVSLLAAASYFTPVLSSALAAFLLSAALSWSFWQGAAMVCGGSLLCWYATRRP

SEQ ID NO: 6 - DNA, 371 bp, synthetic construct
  misc_feature 1..371: note = synthetic_Kcr gene encoding Kcr protein
  source 1..371: mol_type = other DNA
atggataagaaaagagcgacgctcattggatttagcgccattattttgtggagtacgatggtgggtctgattcgcggcgtaagcgaagggctcggcccggtgggcggagccgcaatgatttacagcctcagcggcctgctgctgatttttaccgttggcttcccacaattgcgccaaattccaccgcgctatttgctggtaggtagcctgttttttgtcagctacgaaatgtgcctcgcgctctcattaggctatgccggcactcgccaacaggccatcgaagtcggcatggtgaattatctctggcctagcctgacgattttatttgcgattatctttaatggtcaaaaaaccacctggctggttatccc

SEQ ID NO: 7 - protein, 238 aa, synthetic construct
  REGION 1..238: note = synthetic_Cst protein
MSTLSILIAGFALGLSLIVAIGPQNALLIKQGIKREHVWVVIAICAVSDIILISGGTAGVGYLVETFPTALVVLKYLGAIYLAYFTYLCFRDALRDKVETLSPAQIEPNKTQQIDAFDGGDLGGSSVDTRRRTTRLRQQVRQSTWVKPALATLAICWLNPAAYVDVLVMIGGLANQYGETGRWFFAAGAIAASMLWFPSVGLAAAKFSHVLSRPAVWRGINFGIGCIMALLTIKLLLT

SEQ ID NO: 8 - DNA, 717 bp, synthetic construct
  misc_feature 1..717: note = synthetic_Cst gene encoding Cst protein
  source 1..717: mol_type = other DNA
atgtcaacgctgtctatcctcatcgccggtttcgcactagggctctcacttatcgtagcgattggcccgcaaaatgctctgctgatcaaacagggcattaaacgcgagcacgtgtgggtagtcattgcgatttgcgcggtgtccgacattattttgattagcggtggcaccgcgggggtgggctatctggtggagactttcccgaccgcactggtggtgctgaagtatctgggcgcgatttatctggcttactttacttatctgtgctttcgcgatgcgttgcgcgacaaggttgaaactctctcccctgcgcagatcgagccgaataagacgcagcagatcgatgcattcgatggcggcgacttgggcggttcttctgttgatacccggcggcgcaccacgcgtctgcgccagcaagtacgccaatcgacctgggtgaagccagctcttgcgaccttggcgatttgctggctgaacccggcagcttatgtcgatgtgctggtaatgattggcggacttgccaaccaatacggcgaaaccggccgatggttttttgctgccggtgccattgcagcgagcatgctgtggtttcccagcgttggtcttgctgccgcgaagttctcgcacgtactttcgcgccctgcggtatggcgcggcatcaacttcggcattggctgcatcatggcgctgctgaccattaagctgctgttgacctag

SEQ ID NO: 9 - protein, 242 aa, synthetic construct
  REGION 1..242: note = synthetic_LsaF protein
MSPSHDPLPRRAGAAAGLRDSLGVGLGIFPLGIALGILVIQAGLPWWLAPALSIGIFAGSVELLLVSMLAAATPLVTIAATVFAVNFRHVFYAFSFPLSRVRPGLPRAYSIYAMIDEAYATYVLMDPDRLSSARMVTGQLAMQLYWVLGGFVGIMIANVLPAPIEGFEFALVALFVVMSMDAIRGKRELPSALLACLAVTVAILVAGDNALLVALALYSGLLGLRYFLTKRTTDTAEEGERA

SEQ ID NO: 10 - protein, 140 aa, synthetic construct
  REGION 1..140: note = synthetic_LsaE protein
MRCWSRLRCTPGYWGCAISSPSEPRTLRRRASVPSTEYLIAGVVVAGLITLALRALPFAALKPLRKSKLVQALGRWMPAGILVILAVVVLRDQLISQQGRVWPVLVATAITALAHLLSKRRALVSIAAGTACYVLLLNFF

SEQ ID NO: 11 - DNA, 1048 bp, synthetic construct
  misc_feature 1..1048: note = synthetic_Isa gene
  source 1..1048: mol_type = other DNA
atgtctccgtcacacgatcctttaccgcgccgcgcgggcgccgcggccggccttcgagattctctcggggtcggcctcggcattttccccttgggcattgccctcggaattcttgtcattcaggcgggacttccctggtggctcgccccggccctctcgattggtatcttcgcgggatctgtcgagctgctcctggtcagcatgctcgccgccgcgactccgctcgtgacgatcgccgcgaccgtgttcgccgtgaactttcggcacgtattctacgcgttctcgtttccgctttcgcgggtgcgaccgggtctaccccgggcgtactccatctacgcaatgatcgacgaggcctacgccacctatgtgctgatggatccggatcgcctgagctcagcccgcatggtaaccggccagctcgcgatgcagctctattgggtgctcggcggcttcgtcggcatcatgattgcgaacgtgctccctgcccccattgagggctttgagtttgcactcgtggcgctcttcgtggtgatgtcgatggatgcgattcgcggcaagcgcgagctcccatcggccttgctggcttgcctcgctgtcacggttgcaatactggtcgctggcgacaatgcgctgctggtcgcgcttgcgctgtactccgggctactggggctgcgctatttcctcaccaagcgaaccacggacactgcggaggagggcgagcgtgcctagcaccgaatatctaatcgcgggcgtcgtcgtcgcgggcctcatcaccctggcgctgcgcgcactcccgtttgcggcgctcaaaccgctgcgcaaatctaagctcgtgcaggcgctcgggcgctggatgcccgctggcatcctcgttatcctcgccgtcgtcgtactgcgcgatcagctcatatcgcagcagggccgggtgtggccggtgctcgtcgcgaccgcgatcacggccctcgctcacttgctctcaaagcgacgcgcgctcgtgagcatcgcggctggcaccgcctgctacgtgctgctgctcaactttttctag

SEQ ID NO: 12 - protein, 251 aa, synthetic construct
  REGION 1..251: note = synthetic_DvaF protein
MSVEAQPGANDRPYSVRHEITQGALLILPAGLGMIPIGIAFGLLVVQSGLPWWMAPALSFFAYAGSLELLLITLITSLTPLVTIAAASFFVNFRHVFYAFNFPLKVVTNPFLKFYAMYSLTDEIFAVTVANPKGWTQPRVISAGAVLQICWVGGGLMGVLLSSFIPFQIRGLSFALCALFITLTLDACRTKQEIPSLLLGAAAFGFALLLLPSQPIFAAMIGFVATLAARYTIAVRLTRPLPAEMESDDAA

SEQ ID NO: 13 - protein, 111 aa, synthetic construct
  REGION 1..111: note = synthetic_DvaE protein
MQLDIPFWYLASVLLIAFAVTFTLRALPFAILEPLRKSQFVRVMAVWMPAGILVILALATFKSTLAEEPGGLVHLLIASGVTIAVHLFGGRRTLVSVAAGTLAFVLLVNFF

SEQ ID NO: 14 - DNA, 756 bp, synthetic construct
  misc_feature 1..756: note = synthetic_DvaF gene encoding DvaF protein
  source 1..756: mol_type = other DNA
atgagcgttgaggcgcagcctggcgcaaacgaccgaccctatagcgtgcgccacgagatcacgcagggcgcactcctgattctccccgcagggctcggaatgattccgatcggcattgccttcggcctgcttgtggtgcaatcggggctcccgtggtggatggcacccgccctttcgttcttcgcgtacgcgggctcactcgagcttctgctcatcacgctcatcacgtcgcttacgccgcttgtaacgatcgctgcggcatcgttcttcgtgaacttccgccacgtgttctacgcgtttaatttcccgctcaaggtcgtcacgaacccgttcttgaagttctacgcgatgtactccctcaccgacgagatcttcgcggtaacggttgccaatccaaaggggtggacgcagccgcgcgtgatctcggcaggggccgtactccagatctgctgggtgggtggcggcctcatgggggtactgctctcgagcttcatccccttccagatccgcggcctgagtttcgcgctgtgcgccctgttcatcacgctgaccctcgatgcgtgccgcacgaaacaggagatcccgtcacttctcctcggtgctgccgccttcggtttcgcgctccttttgctcccgagccagccgatcttcgccgcgatgattggcttcgtggcgaccctcgccgcgcgctacacgatcgccgtgcgcctcacgaggccactcccggcagagatggagagcgacgatgcagcttga

SEQ ID NO: 15 - DNA, 335 bp, synthetic construct
  misc_feature 1..335: note = synthetic_DvaE gene encoding DvaE protein
  source 1..335: mol_type = other DNA
atgcagcttgacatccccttctggtatctcgcctcggttctcctcatcgccttcgccgtgaccttcacgctgcgcgcgctcccgttcgcgattctcgaaccactgcgcaaatcgcaattcgtgcgcgtcatggccgtgtggatgcccgcgggcatcctcgtgatcctcgcgctcgcgacctttaagagcaccctcgccgaggaacccggtggtctcgttcacctgctgatcgcctcaggagtcacgattgccgtgcacctcttcggtggtcgccgcaccctcgtgagcgtcgccgcgggcaccctcgccttcgtgctgctcgtgaactttttcta

SEQ ID NO: 16 - DNA, 1081 bp, synthetic construct
  misc_feature 1..1081: note = synthetic_DvaFE gene
  source 1..1081: mol_type = other DNA
atgagcgttgaggcgcagcctggcgcaaacgaccgaccctatagcgtgcgccacgagatcacgcagggcgcactcctgattctccccgcagggctcggaatgattccgatcggcattgccttcggcctgcttgtggtgcaatcggggctcccgtggtggatggcacccgccctttcgttcttcgcgtacgcgggctcactcgagcttctgctcatcacgctcatcacgtcgcttacgccgcttgtaacgatcgctgcggcatcgttcttcgtgaacttccgccacgtgttctacgcgtttaatttcccgctcaaggtcgtcacgaacccgttcttgaagttctacgcgatgtactccctcaccgacgagatcttcgcggtaacggttgccaatccaaaggggtggacgcagccgcgcgtgatctcggcaggggccgtactccagatctgctgggtgggtggcggcctcatgggggtactgctctcgagcttcatccccttccagatccgcggcctgagtttcgcgctgtgcgccctgttcatcacgctgaccctcgatgcgtgccgcacgaaacaggagatcccgtcacttctcctcggtgctgccgccttcggtttcgcgctccttttgctcccgagccagccgatcttcgccgcgatgattggcttcgtggcgaccctcgccgcgcgctacacgatcgccgtgcgcctcacgaggccactcccggcagagatggagagcgacgatgcagcttgacatccccttctggtatctcgcctcggttctcctcatcgccttcgccgtgaccttcacgctgcgcgcgctcccgttcgcgattctcgaaccactgcgcaaatcgcaattcgtgcgcgtcatggccgtgtggatgcccgcgggcatcctcgtgatcctcgcgctcgcgacctttaagagcaccctcgccgaggaacccggtggtctcgttcacctgctgatcgcctcaggagtcacgattgccgtgcacctcttcggtggtcgccgcaccctcgtgagcgtcgccgcgggcaccctcgccttcgtgctgctcgtgaactttttctaa

SEQ ID NO: 17 - DNA, 409 bp, synthetic construct
  misc_feature 1..409: note = synthetic_PgapA
  source 1..409: mol_type = other DNA
tctgagactttaatttgtggattcacgggggtgtaatgtagttcataattaaccccattcgggggagcagatcgtagtgcgaacgatttcaggttcgttccctgcaaaaactatttagcgcaagtgttggaaatgcccccgtttggggtcaatgtccatttttgaatgtgtctgtatgattttgcatctgctgcgaaatctttgtttccccgctaaagttgaggacaggttgacacggagttgactcgacgaattatccaatgtgagtaggtttggtgcgtgagttggaaaaattcgccatactcgcccttgggttctgtcagctcaagaattcttgagtgaccgatgctctgattgacctaactgcttgacacattgcatttcctacaatctttagaggagacacaac

SEQ ID NO: 18 - DNA, 40 bp, synthetic construct
  misc_feature 1..40: note = synthetic_primer
  source 1..40: mol_type = other DNA
gtacccggggatcctctagacaaagccgaagagaagttgg

SEQ ID NO: 19 - DNA, 30 bp, synthetic construct
  misc_feature 1..30: note = synthetic_primer
  source 1..30: mol_type = other DNA
gcatagagtactcggcgcccataaatttca

SEQ ID NO: 20 - DNA, 30 bp, synthetic construct
  misc_feature 1..30: note = synthetic_primer
  source 1..30: mol_type = other DNA
gcgccgagtactctatgccgagaagttgaa

SEQ ID NO: 21 - DNA, 40 bp, synthetic construct
  misc_feature 1..40: note = synthetic_primer
  source 1..40: mol_type = other DNA
gcctgcaggtcgactctagactgggcatcacactattttt

SEQ ID NO: 22 - DNA, 531 bp, synthetic construct
  misc_feature 1..531: note = synthetic_del-N2131L
  source 1..531: mol_type = other DNA
gtacccggggatcctctagacaaagccgaagagaagttggcttgacggacccgaaattccagctgattttgacgatcctgatgcacccggcaggtggcctggcgaaaagttggggcttcctcaagaaggggccggctctctgtcctcagtggctcgtcgtatcggcggggtctgcgtggactggggtgtttcctgggttattgctattgtgctgtccaatttcacggatgtgctgggcgatgtagcgacatccacgctcattattttcgtgatcctgggttggcttaccggttggatctttgctcgcaccccaggtcatgccgtgtttggcatgggccttgcgcgtgtggatgcagaggaacgtgtgggctggtggcgtgcgctggttcgcccactgctgacgatcttgattctgcctgccgtgatggtggatgctgacggccgtgggctccacgacaaggcaacgggaactgcagttatccgcgggtaatttgtcttgagtgaaatttatgggcgccgagtactctatgc

SEQ ID NO: 23 - DNA, 555 bp, synthetic construct
  misc_feature 1..555: note = synthetic_del-N2131R
  source 1..555: mol_type = other DNA
gcgccgagtactctatgccgagaagttgaacagcaatcttgcagcaactcctcagtattcacaccagccccaatggacacaaaaacatcagccccagaatcgcccctaagggcctcaaatacacgatctggaccaactagtcatcgggaaaacccaaccccttaaatcgccttctgcgcttaaggggtcaatgctagataagtaggaacaacaacgtttgggcggccaggatctttgcgatcatcgccagcggatacacagaggtataacccatggcagggagctcgttgcgggaggcatctgacacataactcagcacagcagggtgggtttgcgtaccggcgaggatgccagcggtttcaccgaaggggattttcatcagtttgtggccaacgaacagcaccgtgatggagatgaacaaagtgagcagcgcaccgaagccgatgatggtgagtgattgggggtcgctgatcgctgatcgaaatcctgcgcccgctgaggtaccgatggcagccaaaaatagtgtgatgcccagtctagagtcgacctgcaggc

SEQ ID NO: 24 - DNA, 30 bp, synthetic construct
  misc_feature 1..30: note = synthetic_Haq-F
  source 1..30: mol_type = other DNA
aggagacacaacatgaagagcaagaacgca

SEQ ID NO: 25 - DNA, 40 bp, synthetic construct
  misc_feature 1..40: note = synthetic_Haq-R
  source 1..40: mol_type = other DNA
tcaacttctcggcatagagtctattggttctgaggtgggc

SEQ ID NO: 26 - DNA, 40 bp, synthetic construct
  misc_feature 1..40: note = synthetic_PgapA-F
  source 1..40: mol_type = other DNA
gaaatttatgggcgccgagttctgagactttaatttgtgg

SEQ ID NO: 27 - DNA, 30 bp, synthetic construct
  misc_feature 1..30: note = synthetic_PgapA-R
  source 1..30: mol_type = other DNA
cttgctcttcatgttgtgtctcctctaaag

SEQ ID NO: 28 - DNA, 30 bp, synthetic construct
  misc_feature 1..30: note = synthetic_Cpi-F
  source 1..30: mol_type = other DNA
aggagacacaacatgcaaagcacgcgtaag

SEQ ID NO: 29 - DNA, 40 bp, synthetic construct
  misc_feature 1..40: note = synthetic_Cpi-R
  source 1..40: mol_type = other DNA
tcaacttctcggcatagagttcattgcttccagacacggt

SEQ ID NO: 30 - DNA, 30 bp, synthetic construct
  misc_feature 1..30: note = synthetic_PgapA-R
  source 1..30: mol_type = other DNA
cgtgctttgcatgttgtgtctcctctaaag

SEQ ID NO: 31 - DNA, 30 bp, synthetic construct
  misc_feature 1..30: note = synthetic_Kcr-F
  source 1..30: mol_type = other DNA
aggagacacaacatggataagaaaagagcg

SEQ ID NO: 32 - DNA, 40 bp, synthetic construct
  misc_feature 1..40: note = synthetic_Kcr-R
  source 1..40: mol_type = other DNA
tcaacttctcggcatagagtttagggacggcgggtggcgt

SEQ ID NO: 33 - DNA, 30 bp, synthetic construct
  misc_feature 1..30: note = synthetic_PgapA-R
  source 1..30: mol_type = other DNA
tttcttatccatgttgtgtctcctctaaag

SEQ ID NO: 34 - DNA, 30 bp, synthetic construct
  misc_feature 1..30: note = synthetic_Cst-F
  source 1..30: mol_type = other DNA
aggagacacaacatgtcaacgctgtctatc

SEQ ID NO: 35 - DNA, 40 bp, synthetic construct
  misc_feature 1..40: note = synthetic_Cst-R
  source 1..40: mol_type = other DNA
tcaacttctcggcatagagtctaggtcaacagcagcttaa

SEQ ID NO: 36 - DNA, 30 bp, synthetic construct
  misc_feature 1..30: note = synthetic_PgapA-R
  source 1..30: mol_type = other DNA
cagcgttgacatgttgtgtctcctctaaag

SEQ ID NO: 37 - DNA, 30 bp, synthetic construct
  misc_feature 1..30: note = synthetic_Isa-F
  source 1..30: mol_type = other DNA
aggagacacaacatgtctccgtcacacgat

SEQ ID NO: 38 - DNA, 40 bp, synthetic construct
  misc_feature 1..40: note = synthetic_Isa-R
  source 1..40: mol_type = other DNA
tcaacttctcggcatagagtctagaaaaagttgagcagca

SEQ ID NO: 39 - DNA, 30 bp, synthetic construct
  misc_feature 1..30: note = synthetic_PgapA-R
  source 1..30: mol_type = other DNA
tgacggagacatgttgtgtctcctctaaag

SEQ ID NO: 40 - DNA, 30 bp, synthetic construct
  misc_feature 1..30: note = synthetic_Dva-F
  source 1..30: mol_type = other DNA
aggagacacaacatgagcgttgaggcgcag

SEQ ID NO: 41 - DNA, 40 bp, synthetic construct
  misc_feature 1..40: note = synthetic_Dva-R
  source 1..40: mol_type = other DNA
tcaacttctcggcatagagtttagaaaaagttcacgagca

SEQ ID NO: 42 - DNA, 30 bp, synthetic construct
  misc_feature 1..30: note = synthetic_PgapA-R
  source 1..30: mol_type = other DNA
ctcaacgctcatgttgtgtctcctctaaag

SEQ ID NO: 43 - protein, 251 aa, synthetic construct
  REGION 1..251: note = synthetic_HmaF protein
MSVAAQPSAHEHPYSVRHEITQGALLILPAGLGMIPIGIAFGLLVVQSGLPWWMAPALSFFAYAGSLELLLITLITSLTPLVTIAAASFFVNFRHVFYAFNFPLKVVKNPFLKFYAMYSLTDEIFAVTVAHPKGWTQPRVISAGAVLQICWVGGGLMGVLLSSFIPFQIRGLSFALCALFITLTLDACRTKQELPSLVLGAAAFGLALLLMPGQPIFAAMIGFVATLAARYTIAVRLTRPLPAEMEGDDAA

SEQ ID NO: 44 - protein, 111 aa, synthetic construct
  REGION 1..111: note = synthetic_HmaE protein
MQLDIPFWYLASVLLIAFAVTFTLRALPFAILEPLRKSQFVRVMAVWMPAGILVILALATFKSTLAEEPGSVIHLLIASAVTIAVHLLFGRRTLVSVAAGTLAFVLLVNFF

SEQ ID NO: 45 - DNA, 756 bp, synthetic construct
  misc_feature 1..756: note = synthetic_HmaF gene encoding hmaF protein
  source 1..756: mol_type = other DNA
atgagcgttgcggcgcagcctagcgcacatgagcatccctattcggtgcgccatgaaatcacgcagggggcgctcttgattctccccgcgggcctcggcatgatcccgattggcatcgcttttggccttcttgttgtgcagtccggacttccgtggtggatggcacccgccctctcattcttcgcgtacgcgggctcgctcgagcttttgctcatcacactcatcacatcgctcacgccgctcgtgacgatcgctgcggcatcgttcttcgtgaacttccgccacgtgttttacgcgttcaacttcccgctcaaggtcgtgaagaacccgtttttgaagttctacgcgatgtactcgcttaccgacgagatcttcgcggtgacggtcgcgcacccgaaggggtggacgcagccacgcgtcatctccgcgggcgccgtactccagatctgctgggtgggaggcggcctcatgggcgtgctcctctcgagtttcattcccttccagatccgcggtttgagcttcgccctgtgcgcgcttttcatcaccctgactctcgatgcgtgccgcacgaagcaagaacttccgtcgctagttctcggcgccgcggccttcggtctcgccctgctcctcatgcccgggcagccgatctttgccgcgatgatcggcttcgttgcaacgctcgccgcgcggtacacgatcgccgtgcgccttacgaggccgctaccggcggaaatggagggcgacgatgcagcttga

SEQ ID NO: 46 - DNA, 336 bp, synthetic construct
  misc_feature 1..336: note = synthetic_HmaE gene encoding HmaE protein
  source 1..336: mol_type = other DNA
atgcagcttgacatccccttctggtaccttgcctcggttctcctcattgccttcgccgtcacctttacgctgcgcgcgctcccgttcgcgatcctcgaaccgctgcgcaaatcccagttcgtgcgcgtcatggccgtgtggatgcccgcgggcatcctcgtcattctcgcgctcgcgaccttcaaaagcaccctcgctgaggaacccggcagcgtcattcatttgctcattgcctcggccgtcacgatcgctgtgcatcttctctttgggcgccgaaccctcgtgagtgtcgccgcgggtaccctcgccttcgtgctcctcgtgaacttcttctaa

SEQ ID NO: 47 - DNA, 1081 bp, synthetic construct
  misc_feature 1..1081: note = synthetic_HmaFE gene encoding HmaFE protein
  source 1..1081: mol_type = other DNA
atgagcgttgcggcgcagcctagcgcacatgagcatccctattcggtgcgccatgaaatcacgcagggggcgctcttgattctccccgcgggcctcggcatgatcccgattggcatcgcttttggccttcttgttgtgcagtccggacttccgtggtggatggcacccgccctctcattcttcgcgtacgcgggctcgctcgagcttttgctcatcacactcatcacatcgctcacgccgctcgtgacgatcgctgcggcatcgttcttcgtgaacttccgccacgtgttttacgcgttcaacttcccgctcaaggtcgtgaagaacccgtttttgaagttctacgcgatgtactcgcttaccgacgagatcttcgcggtgacggtcgcgcacccgaaggggtggacgcagccacgcgtcatctccgcgggcgccgtactccagatctgctgggtgggaggcggcctcatgggcgtgctcctctcgagtttcattcccttccagatccgcggtttgagcttcgccctgtgcgcgcttttcatcaccctgactctcgatgcgtgccgcacgaagcaagaacttccgtcgctagttctcggcgccgcggccttcggtctcgccctgctcctcatgcccgggcagccgatctttgccgcgatgatcggcttcgttgcaacgctcgccgcgcggtacacgatcgccgtgcgccttacgaggccgctaccggcggaaatggagggcgacgatgcagcttgacatccccttctggtaccttgcctcggttctcctcattgccttcgccgtcacctttacgctgcgcgcgctcccgttcgcgatcctcgaaccgctgcgcaaatcccagttcgtgcgcgtcatggccgtgtggatgcccgcgggcatcctcgtcattctcgcgctcgcgaccttcaaaagcaccctcgctgaggaacccggcagcgtcattcatttgctcattgcctcggccgtcacgatcgctgtgcatcttctctttgggcgccgaaccctcgtgagtgtcgccgcgggtaccctcgccttcgtgctcctcgtgaacttcttctaa

SEQ ID NO: 48 - DNA, 30 bp, synthetic construct
  misc_feature 1..30: note = synthetic_hma-F
  source 1..30: mol_type = other DNA
aggagacacaacatgagcgttgcggcgcag

SEQ ID NO: 49 - DNA, 40 bp, synthetic construct
  misc_feature 1..40: note = synthetic_hma-R
  source 1..40: mol_type = other DNA
tcaacttctcggcatagagtttagaagaagttcacgagga

SEQ ID NO: 50 - DNA, 30 bp, synthetic construct
  misc_feature 1..30: note = synthetic_PgapA-R
  source 1..30: mol_type = other DNA
cgcaacgctcatgttgtgtctcctctaaag

SEQ ID NO: 51 - DNA, 100 bp, synthetic construct
  misc_feature 1..100: note = synthetic_PyccA
  source 1..100: mol_type = other DNA
ttccagatcaaatgcgtaaagatgggtaaaacttctgggtgcccttacgcattatcattatgctgcttaattaattacatctgtcatagagagtgactca

SEQ ID NO: 52 - DNA, 38 bp, synthetic construct
  misc_feature 1..38: note = synthetic_dva-F
  source 1..38: mol_type = other DNA
ctgtcatagagagtgactcaatgagcgttgcggcgcag

SEQ ID NO: 53 - DNA, 40 bp, synthetic construct
  misc_feature 1..40: note = synthetic_dva-R
  source 1..40: mol_type = other DNA
cgggtaccgagctcgaattcttagaagaagttcacgagga

SEQ ID NO: 54 - DNA, 40 bp, synthetic construct
  misc_feature 1..40: note = synthetic_PyccA-F
  source 1..40: mol_type = other DNA
actcactatagggcgaattcttccagatcaaatgcgtaaa

SEQ ID NO: 55 - DNA, 30 bp, synthetic construct
  misc_feature 1..30: note = synthetic_PyccA-R
  source 1..30: mol_type = other DNA
tgagtcactctctatgacagatgtaattaa

SEQ ID NO: 56 - protein, 251 aa, synthetic construct
  REGION 1..251: note = synthetic_HmaF protein (I72L, I124V var.)
MSVAAQPSAHEHPYSVRHEITQGALLILPAGLGMIPIGIAFGLLVVQSGLPWWMAPALSFFAYAGSLELLLLTLITSLTPLVTIAAASFFVNFRHVFYAFNFPLKVVKNPFLKFYAMYSLTDEVFAVTVAHPKGWTQPRVISAGAVLQICWVGGGLMGVLLSSFIPFQIRGLSFALCALFITLTLDACRTKQELPSLVLGAAAFGLALLLMPGQPIFAAMIGFVATLAARYTIAVRLTRPLPAEMEGDDAA